European Patent Specification EP 4 522 635 B1, published July 1, 2026. Title: PEPTIDE HAVING ANTIMICROBIAL ACTIVITY. Applicant: Cabosse Naturals NV. Application WO. The sequence listing filed with the application follows.

SEQUENCE LISTING (23 sequences)

SEQ ID NO: 1 - protein, 56 aa, synthetic construct
  REGION 1..56: note = peptide according to an embodiment of the invention
YGRKQYERDPRQQYEQCQRRCESEATEEREQEQCEQRCEREYKEQQRQQEEELQRQ

SEQ ID NO: 2 - protein, 28 aa, synthetic construct
  REGION 1..28: note = signal peptide according to an embodiment of the invention
MVISKSPFIVLIFSLLLSFALLCSGVSA

SEQ ID NO: 3 - protein, 84 aa, synthetic construct
  REGION 1..84: note = peptide according to an embodiment of the invention
MVISKSPFIVLIFSLLLSFALLCSGVSAYGRKQYERDPRQQYEQCQRRCESEATEEREQEQCEQRCEREYKEQQRQQEEELQRQ

SEQ ID NO: 4 - protein, 47 aa, Theobroma cacao
YERDPRQQYEQCQRRCESEATEEREQEQCEQRCEREYKEQQRQQEEE

SEQ ID NO: 5 - protein, 60 aa, Theobroma cacao
LQRQYQQCQGRCQEQQQGQREQQQCQRKCWEQYKEQERGEHENYHNHKKNRSEEEEGQQR

SEQ ID NO: 6 - DNA, 27 bp, synthetic construct
  misc_feature 1..27: note = Forward_BamH1 forward DNA primer
  source 1..27: mol_type = other DNA
cgcggatcctatggcagaaaacaatat

SEQ ID NO: 7 - DNA, 32 bp, synthetic construct
  misc_feature 1..32: note = Reverse_Kpn1 forward DNA primer
  source 1..32: mol_type = other DNA
ggtacctcattgcctttgaagctcttcttctt

SEQ ID NO: 8 - protein, 6 aa, synthetic construct
  REGION 1..6: note = HQ tag
HQHQHQ

SEQ ID NO: 9 - protein, 12 aa, synthetic construct
  REGION 1..12: note = HN tag
HNHNHNHNHNHN

SEQ ID NO: 10 - protein, 19 aa, synthetic construct
  REGION 1..19: note = HAT tag
KDHLIHNVHKEEHAHAHNK

SEQ ID NO: 11 - protein, 13 aa, synthetic construct
  REGION 1..13: note = ALFA tag
SRLEEELRRRLTE

SEQ ID NO: 12 - protein, 15 aa, synthetic construct
  REGION 1..15: note = Avi tag
GLNDIFEAQKIEWHE

SEQ ID NO: 13 - protein, 4 aa, synthetic construct
  REGION 1..4: note = C-tag
EPEA

SEQ ID NO: 14 - protein, 26 aa, synthetic construct
  REGION 1..26: note = Calmodulin-tag
KRRWKKNFIAVSAANRFKKISSSGAL

SEQ ID NO: 15 - protein, 13 aa, synthetic construct
  REGION 1..13: note = E-tag
GAPVPYPDPLEPR

SEQ ID NO: 16 - protein, 8 aa, synthetic construct
  REGION 1..8: note = FLAG-tag
DYKDDDDK

SEQ ID NO: 17 - protein, 9 aa, synthetic construct
  REGION 1..9: note = HA-tag
YPYDVPDYA

SEQ ID NO: 18 - protein, 10 aa, synthetic construct
  REGION 1..10: note = Myc-tag
EQKLISEEDL

SEQ ID NO: 19 - protein, 18 aa, synthetic construct
  REGION 1..18: note = NE-tag
TKENPRSNQEESYDDNES

SEQ ID NO: 20 - protein, 9 aa, synthetic construct
  REGION 1..9: note = Rho1D4 tag
TETSQVAPA

SEQ ID NO: 21 - protein, 15 aa, synthetic construct
  REGION 1..15: note = S-tag
KETAAAKFERQHMDS

SEQ ID NO: 22 - protein, 37 aa, synthetic construct
  REGION 1..37: note = SBP tag
DEKTTGWRGGHVVEGLAGELEQLRARLEHHPQGQREP

SEQ ID NO: 23 - protein, 8 aa, synthetic construct
  REGION 1..8: note = Strep-tag
WSHPQFEK